European Patent Specification EP 3 291 824 B1, published November 5, 2025. Title: ANTIMICROBIAL THERAPY. Applicant: The Regents of the University of California Nakatsuji, Teruaki Gallo, Richard L. Application Not yet assigned. The sequence listing filed with the application follows.

SEQUENCE LISTING (55 sequences)

SEQ ID NO: 1 - DNA, 186 bp, Staphylococcus hominis
  CDS (1)..(186)
atgagtaaattagaactacttaatgaatctaaagcaaattatcttgaaaaacttactgatgaaaaaattgaagaaacggaagcatacggcggtaaatgttcttggtggaatgcatcatgtcatttaggaaataatgggaaaatttgtacagtttctcatgagtgtgcagcaggatgtaatttataa

SEQ ID NO: 2 - protein, 61 aa, Staphylococcus hominis
MSKLELLNESKANYLEKLTDEKIEETEAYGGKCSWWNASCHLGNNGKICTVSHECAAGCNL

SEQ ID NO: 3 - DNA, 201 bp, Staphylococcus hominis
  CDS (1)..(201)
atgtttagtaaaaatttccaaagaaatgaaaagatggaaaatactttgaaaaaggtaagttcagctaatgatgtgaatggaggagctacaccgactattactacatcttcagcaacttgtggtggtattattgttgcggcaagtgctgctcagtgtccgacattagcttgctcttctagatgtggaaaaagaaaaaaataa

SEQ ID NO: 4 - protein, 66 aa, Staphylococcus hominis
MFSKNFQRNEKMENTLKKVSSANDVNGGATPTITTSSATCGGIIVAASAAQCPTLACSSRCGKRKK

SEQ ID NO: 5 - protein, 170 aa, Homo sapiens
MKTQRNGHSLGRWSLVLLLLGLVMPLAIIAQVLSYKEAVLRAIDGINQRSSDANLYRLLDLDPRPTMDGDPDTPKPVSFTVKETVCPRTTQQSPEDCDFKKDGLVKRCMGTVTLNQARGSFDISCDKDNKRFALLGDFFRKSKEKIGKEFKRIVQRIDDFLRNLVPRTES

SEQ ID NO: 6 - protein, 5 aa, Artificial Sequence
  Synthetic linker
GGGGS

SEQ ID NO: 7 - protein, 22 aa, Artificial Sequence
  Synthetic linker
GGGGGGSMFGGAKKRSGGGGGG

SEQ ID NO: 8 - DNA, 20 bp, Artificial Sequence
  Staphylococcus aureus-specific PCR primer
aactgttggccactatgagt

SEQ ID NO: 9 - DNA, 21 bp, Artificial Sequence
  Staphylococcus aureus-specific PCR primer
ccagcattacctgtaatctcg

SEQ ID NO: 10 - DNA, 20 bp, Artificial Sequence
  Staphylococcus epidermidis-specific PCR primer
tcagcagttgaaggacagat

SEQ ID NO: 11 - DNA, 22 bp, Artificial Sequence
  Staphylococcus epidermidis-specific PCR primer
ccagaacaatgaatggttaagg

SEQ ID NO: 12 - DNA, 30 bp, Artificial Sequence
  Staphylococcus-genus specific 16S sequence PCR primer
tttgggctacacacgtgctacaatggacaa

SEQ ID NO: 13 - DNA, 24 bp, Artificial Sequence
  Staphylococcus-genus specific 16S sequence PCR primer
aacaactttatgggatttgcwtga

SEQ ID NO: 14 - DNA, 21 bp, Artificial Sequence
  Universal sequence of bacterial 16S rRNA PCR primer
agagtttggatcmtggctcag

SEQ ID NO: 15 - DNA, 17 bp, Artificial Sequence
  Universal sequence of bacterial 16S rRNA PCR primer
aaggaggtgwtccarcc

SEQ ID NO: 16 - DNA, 21 bp, Artificial Sequence
  Staphylococcus epidermidis epidermn PCR primer
gattcaggagctgaaccaaga

SEQ ID NO: 17 - DNA, 20 bp, Artificial Sequence
  Staphylococcus epidermidis epidermn PCR primer
ttgaagccctgccaatctaa

SEQ ID NO: 18 - DNA, 24 bp, Artificial Sequence
  Staphylococcus epidermidis pep5 PCR primer
ctgatgaacttgaacctcaaactg

SEQ ID NO: 19 - DNA, 23 bp, Artificial Sequence
  Staphylococcus epidermidis pep5 PCR primer
gacactgtaaataaacgcgtagc

SEQ ID NO: 20 - DNA, 24 bp, Artificial Sequence
  Staphylococcus epidermidis epicidin280 PCR primer
gcaactagacaggtatgtcctaaa

SEQ ID NO: 21 - DNA, 25 bp, Artificial Sequence
  Staphylococcus epidermidis epicidin280 PCR primer
catctaagattaaatgagggtggtt

SEQ ID NO: 22 - DNA, 21 bp, Artificial Sequence
  Staphylococcus epidermidis epilancin K7 PCR primer
taagtccgcaatctgctagtg

SEQ ID NO: 23 - DNA, 22 bp, Artificial Sequence
  Staphylococcus epidermidis epilancin K7 PCR primer
cagtaatattgcaaccgcatgt

SEQ ID NO: 24 - DNA, 25 bp, Artificial Sequence
  Staphylococcus hominis Hogocidin-alpha PCR primer
atgagtaaattagaactacttaatg

SEQ ID NO: 25 - DNA, 25 bp, Artificial Sequence
  Staphylococcus hominis Hogocidin-alpha PCR primer
ttataaattacatcctgctgcacac

SEQ ID NO: 26 - protein, 8 aa, Staphylococcus hominis
KCSDDNAA

SEQ ID NO: 27 - DNA, 138 bp, Staphylococcus hominis
  CDS (1)..(138)
atggatattataaaagtaaataaaacagaaagaatgaatgataatagaaaaattgtaatgattttttctttatacgatacattttttaacgctactaatacacataagctaaagagtatgaagcttaatgcgaaataa

SEQ ID NO: 28 - protein, 45 aa, Staphylococcus hominis
MDIIKVNKTERMNDNRKIVMIFSLYDTFFNATNTHKLKSMKLNAK

SEQ ID NO: 29 - DNA, 168 bp, Staphylococcus epidermidis
  CDS (1)..(168)
atggtatggatccatggtggtggtaacttaggtggtgctggcttagaagatgcttttgatggtaatactttagctaaacatacatcaaaaattaaatatgtttttggaaatttgcaacctgaaaaccattatgatgatattgatataataatctcaaaacaattataa

SEQ ID NO: 30 - protein, 55 aa, Staphylococcus epidermidis
MVWIHGGGNLGGAGLEDAFDGNTLAKHTSKIKYVFGNLQPENHYDDIDIIISKQL

SEQ ID NO: 31 - DNA, 207 bp, Staphylococcus epidermidis
  CDS (1)..(207)
atgatttcagtgatactgccgatggaagaaataattattgcaataataaataacgacttaggccatttaatttttgagaataaaaaaaatagtgggttttcttttttcataataaaacctttcataactaatatttattttctatcaggtattaaaaaaattttacaaaaacagagaaaatattatacgatgctaataaaagtataa

SEQ ID NO: 32 - protein, 68 aa, Staphylococcus epidermidis
MISVILPMEEIIIAIINNDLGHLIFENKKNSGFSFFIIKPFITNIYFLSGIKKILQKQRKYYTMLIKV

SEQ ID NO: 33 - DNA, 210 bp, Staphylococcus epidermidis
  CDS (1)..(210)
atgaacatatacttaaaagtaattttaacttctttattttttgctttaataatttttattgtaacttatataacgactaagcaatggggaacatcgttaggtttttcatctttatcatttatcggtaactttatttacgattattcaacgaaattaagtgataaaaaatatgaaaaaagaataaatagcaacaaaaaagataaactttag

SEQ ID NO: 34 - protein, 69 aa, Staphylococcus epidermidis
MNIYLKVILTSLFFALIIFIVTYITTKQWGTSLGFSSLSFIGNFIYDYSTKLSDKKYEKRINSNKKDKL

SEQ ID NO: 35 - DNA, 183 bp, Staphylococcus epidermidis
  CDS (1)..(183)
atgaaaaataacaaaaatttatttgatttagaaattaaaaaagaaacaagtcaaaacactgatgaacttgaacctcaaactgctggaccagcgattagagcttctgtgaaacaatgtcagaaaactttgaaagctacgcgtttatttacagtgtcttgcaaaggaaaaaacggatgtaaatag

SEQ ID NO: 36 - protein, 60 aa, Staphylococcus epidermidis
MKNNKNLFDLEIKKETSQNTDELEPQTAGPAIRASVKQCQKTLKATRLFTVSCKGKNGCK

SEQ ID NO: 37 - DNA, 171 bp, Staphylococcus hominis
  CDS (1)..(171)
atggaaaacaaaaaagatttatttgatttagaaatcaaaaaagataatatggaaaataataatgaattagaagctcaatctcttggtcctgcaattaaggcaactagacaggtatgtcctaaagcaacacgttttgttacagtttcttgtaaaaaaagtgattgtcaatag

SEQ ID NO: 38 - protein, 56 aa, Staphylococcus hominis
MENKKDLFDLEIKKDNMENNNELEAQSLGPAIKATRQVCPKATRFVTVSCKKSDCQ

SEQ ID NO: 39 - DNA, 135 bp, Staphylococcus hominis
  CDS (1)..(135)
atgaaagttgttaaagaaaagaaagaactttttgatcttgacgttaaagtaaatgcgagagacatgaataattcagaatcaggtccacctaatacaagtttaatatggtgtacggatggatgcgctaaacggtaa

SEQ ID NO: 40 - protein, 44 aa, Staphylococcus hominis
MKVVKEKKELFDLDVKVNARDMNNSESGPPNTSLIWCTDGCAKR

SEQ ID NO: 41 - DNA, 138 bp, Staphylococcus hominis; identical to SEQ ID NO: 27
  CDS (1)..(138)

SEQ ID NO: 42 - protein, 45 aa, Staphylococcus hominis; identical to SEQ ID NO: 28

SEQ ID NO: 43 - DNA, 201 bp, Staphylococcus hominis
  CDS (1)..(201)
atgagtaataaagatttagaattatttaatacagccggtgatttaatacaagaattaaaagatggtgacctaaatatccatttatatggtgaatcggaaattagaaaaaaatctttctctcaaaaaacagggaatgatgggaaacattgtacaattacttgggaatgttctatatgtcctactaaaacttgttggtgctaa

SEQ ID NO: 44 - protein, 66 aa, Staphylococcus hominis
MSNKDLELFNTAGDLIQELKDGDLNIHLYGESEIRKKSFSQKTGNDGKHCTITWECSICPTKTCWC

SEQ ID NO: 45 - DNA, 117 bp, Staphylococcus hominis
  CDS (1)..(117)
atgggaacttcagaggtaagaaaaggaaaaggaggcggttttagtaccgtaaccgttgtaacaccaattgtaccgacatcgaagtgtgcctcaattgtaaaaccatgtaacaaataa

SEQ ID NO: 46 - protein, 38 aa, Staphylococcus hominis
MGTSEVRKGKGGGFSTVTVVTPIVPTSKCASIVKPCNK

SEQ ID NO: 47 - DNA, 165 bp, Staphylococcus hominis
  CDS (1)..(165)
atgactaaaataactaaagatgatttgaaaaagattacagaaaatcgtattgaagcacgtacacatccaaccgttgttcctgtaagtgctgctgtatgcggagttgctactaaattagtaccaacatcgaaatgtgcttcaattgtaaaaccatgtaataaataa

SEQ ID NO: 48 - protein, 54 aa, Staphylococcus hominis
MTKITKDDLKKITENRIEARTHPTVVPVSAAVCGVATKLVPTSKCASIVKPCNK

SEQ ID NO: 49 - DNA, 522 bp, Staphylococcus hominis
  CDS (1)..(522)
atgactatagatttagtaatgatacttattattttgatgtatatgataattggttttagaagaggcctttggctgaatagtcttcatttgtcgtctacacttgtctcactattcattgcgcatcgtttttaccaatatatatcaaaacaaatgattgtttttgttccatttcctaaaacagttgcttttgacacgcacttcgcatttcaataccatgatgtacaacaacgttttgatactattgtggcatttttatgtattgcttttataagtaagttgcttttatatcttattattgtaacttttgataatatagtgtcatatcataatattcatgttacaagtcgaatattgggaagcgtattaggtagtattgcaagtgtgattgtactgcaacttgttttatatttagtatctttatatcctaatgaatggattcaagaaagtttaaaatacggttatttaagccatattattctatttaagatgccgtttttatcatcttatatactaaatttataa

SEQ ID NO: 50 - protein, 173 aa, Staphylococcus hominis
MTIDLVMILIILMYMIIGFRRGLWLNSLHLSSTLVSLFIAHRFYQYISKQMIVFVPFPKTVAFDTHFAFQYHDVQQRFDTIVAFLCIAFISKLLLYLIIVTFDNIVSYHNIHVTSRILGSVLGSIASVIVLQLVLYLVSLYPNEWIQESLKYGYLSHIILFKMPFLSSYILNL

SEQ ID NO: 51 - DNA, 522 bp, Staphylococcus epidermidis
  CDS (1)..(522)
atgctcattgatatagttgttcttcttattatttgttactttatagtgatagggtttcgtagaggtatttggttatcgatattgcactttgcttcttcaattgtatctttatatattgcgtcacaacattatcaatcgattgcgcaacgtttagttgtatttgtgccatttccgaaaacggtggcgtttgatatggtctatactataccttatgatcatttgcaatacagatttgaaaaagtgatagcatttattataatatttggtatgtgtaagcttattttgtatctagttgttgttacatttgataatataataacgtataaaaagatacatttagtaagtcggatatcgagtgtcgttttgagtatcatatcggtttttatatatttacaaattggactttatttattatcgctatatccgcattcatttatacagtaccaattatctcaatcgctagtaagtcgagttgtgattgaacaaattccttatttatcacaatttattttaaatttataa

SEQ ID NO: 52 - protein, 173 aa, Staphylococcus epidermidis
MLIDIVVLLIICYFIVIGFRRGIWLSILHFASSIVSLYIASQHYQSIAQRLVVFVPFPKTVAFDMVYTIPYDHLQYRFEKVIAFIIIFGMCKLILYLVVVTFDNIITYKKIHLVSRISSVVLSIISVFIYLQIGLYLLSLYPHSFIQYQLSQSLVSRVVIEQIPYLSQFILNL

SEQ ID NO: 53 - DNA, 1260 bp, Staphylococcus epidermidis
  CDS (1)..(1260)
atgattggtagaaaaaaagaaacccttttaaaaaacgaagttatttctgcgtttactactttttttacctgcagttatataataattgttaatggtatattgttacatcaagcaggaatgtctttgttatggacgattatagctactactctagtttgttgcattagttgcatccttcttggtatatatgctaatgttccactaattattataccaggaatcggtgaaactattttttttacttatacaatcattaaaagtcattactataattatcatgaagcgctagctattgttttgatttcaggtttgattttcacttttattgcatacacaccgtttgctagagttctagacaagtccataccaaagaatttaaaagaaggaataactattggtataggtctgtttatggcgtttgttggactacaaaacagcaaaataattataccaaacaggcaaagtattgttgagctaaaccacataaacatttatagtgggttagcgatactactactattatttgcaattgttatatttactttagggaccaagttggctttcttttatacagtaattattggtatcattatatcttttttagctgggattataaaggtgaaatatcatttttataattttagtttgcgatcaatagtaagcgagaataatatttttagttacagttttgataaaataggtcatttttctttttggtctttagtgttctcacttactattttgttactgtttcaaaatttaggtacattacatggattgaaaattaatgataaagtaaaattgtcaagaatttttaaaatggtcggtattactaacataatttcaagcttatttggtgtgagttctacagttattgcagtcgaaagttctactgcaactcattcaggagctaaaacaggaaaagtatctatttttgtaggtataatgtttcttttatctttgttgataatgcccgttattatagcaatacctagtttagttgtatcacctatcttaataattgttggcggtttaatgtttactaatattaaagaattagattttaatgatatgactgaatttattccttgttatataacaattataatgataccacttacttttgatattgcaactggaatgggatttggatttatttcatatgttctaattaattttgtatgcaaaaaaaccgaacgtttaaatccaattttaataattattgctttactttttacaataaatttagttttacaataa

SEQ ID NO: 54 - protein, 419 aa, Staphylococcus epidermidis
MIGRKKETLLKNEVISAFTTFFTCSYIIIVNGILLHQAGMSLLWTIIATTLVCCISCILLGIYANVPLIIIPGIGETIFFTYTIIKSHYYNYHEALAIVLISGLIFTFIAYTPFARVLDKSIPKNLKEGITIGIGLFMAFVGLQNSKIIIPNRQSIVELNHINIYSGLAILLLLFAIVIFTLGTKLAFFYTVIIGIIISFLAGIIKVKYHFYNFSLRSIVSENNIFSYSFDKIGHFSFWSLVFSLTILLLFQNLGTLHGLKINDKVKLSRIFKMVGITNIISSLFGVSSTVIAVESSTATHSGAKTGKVSIFVGIMFLLSLLIMPVIIAIPSLVVSPILIIVGGLMFTNIKELDFNDMTEFIPCYITIIMIPLTFDIATGMGFGFISYVLINFVCKKTERLNPILIIIALLFTINLVLQ

SEQ ID NO: 55 - protein, 10 aa, Staphylococcus epidermidis
  MISC_FEATURE (10)..(10): Xaa at 10 is V or L
KNGAYKAQGX